European Patent Application EP 4 570 260 A1, published June 18, 2025. Title: Viral vector for transfection of adipocytes. Applicant: Medizinische Hochschule Hannover. Application EP. The sequence listing filed with the application follows.

SEQUENCE LISTING (82 sequences)

SEQ ID NO: 1 - protein, 7 aa, synthetic construct
NFEELVI

SEQ ID NO: 2 - protein, 7 aa, synthetic construct
LETFLGF

SEQ ID NO: 3 - protein, 7 aa, synthetic construct
WDVLVGA

SEQ ID NO: 4 - protein, 7 aa, synthetic construct
FLDFVSG

SEQ ID NO: 5 - protein, 7 aa, synthetic construct
LDSLLLC

SEQ ID NO: 6 - protein, 7 aa, synthetic construct
LLGFGDM

SEQ ID NO: 7 - protein, 7 aa, synthetic construct
VASLLWD

SEQ ID NO: 8 - protein, 7 aa, synthetic construct
ISLLMNH

SEQ ID NO: 9 - protein, 7 aa, synthetic construct
LAAIFQS

SEQ ID NO: 10 - protein, 7 aa, synthetic construct
FIPVGVS

SEQ ID NO: 11 - protein, 7 aa, synthetic construct
LDLLFVS

SEQ ID NO: 12 - protein, 7 aa, synthetic construct
FLSVLGT

SEQ ID NO: 13 - protein, 7 aa, synthetic construct
GNKTTDR

SEQ ID NO: 14 - protein, 7 aa, synthetic construct
FSELWDT

SEQ ID NO: 15 - protein, 7 aa, synthetic construct
MVLEALC

SEQ ID NO: 16 - protein, 7 aa, synthetic construct
LLQFMTS

SEQ ID NO: 17 - protein, 7 aa, synthetic construct
KPTVDIW

SEQ ID NO: 18 - protein, 7 aa, synthetic construct
FGYVDGK

SEQ ID NO: 19 - protein, 7 aa, synthetic construct
YDIIFDR

SEQ ID NO: 20 - protein, 7 aa, synthetic construct
VLFLASD

SEQ ID NO: 21 - protein, 7 aa, synthetic construct
LDSLLLC

SEQ ID NO: 22 - protein, 7 aa, synthetic construct
NFEELVI

SEQ ID NO: 23 - protein, 7 aa, synthetic construct
SVGSLFC

SEQ ID NO: 24 - protein, 7 aa, synthetic construct
FRTNSGV

SEQ ID NO: 25 - protein, 7 aa, synthetic construct
SVYDNLC

SEQ ID NO: 26 - protein, 7 aa, synthetic construct
FKGGDYF

SEQ ID NO: 27 - protein, 7 aa, synthetic construct
SNSLFNP

SEQ ID NO: 28 - protein, 7 aa, synthetic construct
NMGEEFW

SEQ ID NO: 29 - protein, 7 aa, synthetic construct
FGYVDGK

SEQ ID NO: 30 - protein, 7 aa, synthetic construct
SQTLGLF

SEQ ID NO: 31 - protein, 7 aa, synthetic construct
TSLGQVT

SEQ ID NO: 32 - protein, 7 aa, synthetic construct
IGWPDVS

SEQ ID NO: 33 - protein, 7 aa, synthetic construct
FGPNMLC

SEQ ID NO: 34 - protein, 7 aa, synthetic construct
SLNAVYS

SEQ ID NO: 35 - protein, 7 aa, synthetic construct
SFCDFPD

SEQ ID NO: 36 - protein, 7 aa, synthetic construct
DFSLFAC

SEQ ID NO: 37 - protein, 7 aa, synthetic construct
LYAEKLA

SEQ ID NO: 38 - protein, 7 aa, synthetic construct
ILDKALN

SEQ ID NO: 39 - protein, 7 aa, synthetic construct
LLEGVIC

SEQ ID NO: 40 - protein, 7 aa, synthetic construct
FDTSIFC

SEQ ID NO: 41 - protein, 7 aa, synthetic construct
SSQSSPF

SEQ ID NO: 42 - protein, 7 aa, synthetic construct
MSPFVAG

SEQ ID NO: 43 - protein, 7 aa, synthetic construct
SDRAVSR

SEQ ID NO: 44 - protein, 7 aa, synthetic construct
SLQRGVG

SEQ ID NO: 45 - protein, 7 aa, synthetic construct
SAGSVRV

SEQ ID NO: 46 - protein, 7 aa, synthetic construct
GDRSSRL

SEQ ID NO: 47 - protein, 7 aa, synthetic construct
NDRLHSR

SEQ ID NO: 48 - protein, 7 aa, synthetic construct
TQTFVVG

SEQ ID NO: 49 - protein, 7 aa, synthetic construct
NRARSCT

SEQ ID NO: 50 - protein, 7 aa, synthetic construct
SGLRSMG

SEQ ID NO: 51 - protein, 7 aa, synthetic construct
GSETRKG

SEQ ID NO: 52 - protein, 7 aa, synthetic construct
VDKRRHY

SEQ ID NO: 53 - protein, 7 aa, synthetic construct
SQVGPFK

SEQ ID NO: 54 - protein, 7 aa, synthetic construct
KLGPTSR

SEQ ID NO: 55 - protein, 7 aa, synthetic construct
LPVAASR

SEQ ID NO: 56 - protein, 7 aa, synthetic construct
GVELPLE

SEQ ID NO: 57 - protein, 7 aa, synthetic construct
VGSSTVR

SEQ ID NO: 58 - protein, 7 aa, synthetic construct
SSKAGMR

SEQ ID NO: 59 - protein, 7 aa, synthetic construct
EGVSVRR

SEQ ID NO: 60 - protein, 7 aa, synthetic construct
SGGTGMR

SEQ ID NO: 61 - protein, 7 aa, synthetic construct
KSFALKN

SEQ ID NO: 62 - protein, 7 aa, synthetic construct
SDRAVSR

SEQ ID NO: 63 - protein, 7 aa, synthetic construct
SGMGYLM

SEQ ID NO: 64 - protein, 7 aa, synthetic construct
KAVGTWT

SEQ ID NO: 65 - protein, 7 aa, synthetic construct
IESVRVR

SEQ ID NO: 66 - protein, 7 aa, synthetic construct
ETLWAVS

SEQ ID NO: 67 - protein, 7 aa, synthetic construct
EGTTFDW

SEQ ID NO: 68 - protein, 7 aa, synthetic construct
SRFGVPS

SEQ ID NO: 69 - protein, 7 aa, synthetic construct
FASGALG

SEQ ID NO: 70 - protein, 7 aa, synthetic construct
VKKGGLS

SEQ ID NO: 71 - protein, 7 aa, synthetic construct
SSALARS

SEQ ID NO: 72 - protein, 7 aa, synthetic construct
EGNRPSR

SEQ ID NO: 73 - protein, 7 aa, synthetic construct
KGTVAGR

SEQ ID NO: 74 - protein, 7 aa, synthetic construct
KAAAVNR

SEQ ID NO: 75 - protein, 7 aa, synthetic construct
VCGMGIR

SEQ ID NO: 76 - protein, 7 aa, synthetic construct
TGCARGS

SEQ ID NO: 77 - protein, 7 aa, synthetic construct
GNANLRK

SEQ ID NO: 78 - protein, 7 aa, synthetic construct
SLRGSGS

SEQ ID NO: 79 - protein, 7 aa, synthetic construct
NAAASVS

SEQ ID NO: 80 - protein, 7 aa, synthetic construct
GNAGPRK

SEQ ID NO: 81 - protein, 736 aa, Adeno-associated dependoparvovirus A
  CHAIN 1..736: note = capsid protein
MAADGYLPDWLEDNLSEGIREWWDLKPGAPKPKANQQKQDDGRGLVLPGYKYLGPFNGLDKGEPVNAADAAALEHDKAYDQQLKAGDNPYLRYNHADAEFQERLQEDTSFGGNLGRAVFQAKKRVLEPLGLVEEGAKTAPGKKRPVEQSPQEPDSSSGIGKTGQQPAKKRLNFGQTGDSESVPDPQPLGEPPATPAAVGPTTMASGGGAPMADNNEGADGVGNASGNWHCDSTWLGDRVITTSTRTWALPTYNNHLYKQISSASTGASNDNHYFGYSTPWGYFDFNRFHCHFSPRDWQRLINNNWGFRPKRLNFKLFNIQVKEVTTNDGVTTIANNLTSTVQVFSDSEYQLPYVLGSAHQGCLPPFPADVFMIPQYGYLTLNNGSQAVGRSSFYCLEYFPSQMLRTGNNFTFSYTFEEVPFHSSYAHSQSLDRLMNPLIDQYLYYLNRTQNQSGSAQNKDLLFSRGSPAGMSVQPKNWLPGPCYRQQRVSKTKTDNNNSNFTWTGASKYNLNGRESIINPGTAMASHKDDEDKFFPMSGVMIFGKESAGASNTALDNVMITDEEEIKATNPVATERFGTVAVNFQSSSTDPATGDVHAMGALPGMVWQDRDVYLQGPIWAKIPHTDGHFHPSPLMGGFGLKNPPPQILIKNTPVPANPPAEFSATKFASFITQYSTGQVSVEIEWELQKENSKRWNPEVQYTSNYAKSANVDFTVDNNGLYTEPRPIGTRYLTRPL

SEQ ID NO: 82 - protein, 748 aa, synthetic construct
  CHAIN 1..590: note = section of wild-type capsid
  CHAIN 591..593: note = linker
  CHAIN 601..602: note = linker
  UNSURE 594: note = any one of A, R, N, D, C, Q, E, G, H, I, L, K, M, F, P, O, S, U, T, W, Y, or V
  UNSURE 595: note = any one of A, R, N, D, C, Q, E, G, H, I, L, K, M, F, P, O, S, U, T, W, Y, or V
  UNSURE 596: note = any one of A, R, N, D, C, Q, E, G, H, I, L, K, M, F, P, O, S, U, T, W, Y, or V
  UNSURE 597: note = any one of A, R, N, D, C, Q, E, G, H, I, L, K, M, F, P, O, S, U, T, W, Y, or V
  UNSURE 598: note = any one of A, R, N, D, C, Q, E, G, H, I, L, K, M, F, P, O, S, U, T, W, Y, or V
  UNSURE 599: note = any one of A, R, N, D, C, Q, E, G, H, I, L, K, M, F, P, O, S, U, T, W, Y, or V
  UNSURE 600: note = any one of A, R, N, D, C, Q, E, G, H, I, L, K, M, F, P, O, S, U, T, W, Y, or V
  CHAIN 603..748: note = section of wild-type capsid
MAADGYLPDWLEDNLSEGIREWWDLKPGAPKPKANQQKQDDGRGLVLPGYKYLGPFNGLDKGEPVNAADAAALEHDKAYDQQLKAGDNPYLRYNHADAEFQERLQEDTSFGGNLGRAVFQAKKRVLEPLGLVEEGAKTAPGKKRPVEQSPQEPDSSSGIGKTGQQPAKKRLNFGQTGDSESVPDPQPLGEPPATPAAVGPTTMASGGGAPMADNNEGADGVGNASGNWHCDSTWLGDRVITTSTRTWALPTYNNHLYKQISSASTGASNDNHYFGYSTPWGYFDFNRFHCHFSPRDWQRLINNNWGFRPKRLNFKLFNIQVKEVTTNDGVTTIANNLTSTVQVFSDSEYQLPYVLGSAHQGCLPPFPADVFMIPQYGYLTLNNGSQAVGRSSFYCLEYFPSQMLRTGNNFTFSYTFEEVPFHSSYAHSQSLDRLMNPLIDQYLYYLNRTQNQSGSAQNKDLLFSRGSPAGMSVQPKNWLPGPCYRQQRVSKTKTDNNNSNFTWTGASKYNLNGRESIINPGTAMASHKDDEDKFFPMSGVMIFGKESAGASNTALDNVMITDEEEIKATNPVATERFGTVAVNFQSSSTDAAAXXXXXXXAAPATGDVHAMGALPGMVWQDRDVYLQGPIWAKIPHTDGHFHPSPLMGGFGLKNPPPQILIKNTPVPANPPAEFSATKFASFITQYSTGQVSVEIEWELQKENSKRWNPEVQYTSNYAKSANVDFTVDNNGLYTEPRPIGTRYLTRPL